European Patent Application EP 4 235 676 A2, published August 30, 2023. Title: METHODS FOR NON-INVASIVE ASSESSMENT OF GENETIC ALTERATIONS. Applicant: Sequenom, Inc. Application EP. The sequence listing filed with the application follows.

SEQUENCE LISTING (2 sequences)

SEQ ID NO: 1 - DNA, 18 bp, synthetic construct
  misc_feature 1..18: note = Synthetic construct
  source 1..18: mol_type = other DNA
tgattcaagcattcgatc

SEQ ID NO: 2 - DNA, 18 bp, synthetic construct
  misc_feature 1..18: note = Synthetic construct
  source 1..18: mol_type = other DNA
gggtgcccccaaaatatt